European Patent Specification EP 4 063 392 B1, published July 30, 2025. Title: ANTI-TUMOR ANTIGEN NANOBODY AND NUCLEIC ACID ENCODING SEQUENCE THEREOF, AND USES OF THE SAME. Applicant: CHINA MEDICAL UNIVERSITY HOSPITAL. The sequence listing filed with the application follows.

SEQUENCE LISTING (15 sequences)

SEQ ID NO: 1 - protein, 133 aa, Artificial Sequence
  anti-HLA-G nanobody clone#9
MGQVQLVESGGGSVQAGGSLRLSCEASGRTYSSNCMGWFRQAPGKERENVAAIYTGGDGITYADSVKGRFTISQDKLKNMLYLQMDSLKPEDTAMYYCAADPNRRRMGVGGSCLRANFGPGGQGTQVTVSSLE

SEQ ID NO: 2 - protein, 117 aa, Artificial Sequence
  anti-HLA-G nanobody clone#20
EVQLVESGGGSVRPGETLRLSCTASGFTVDDSDMSWYRQAPGDECELVSSITSGGGKYYSHPVKGRFTIFRDKGKNTMYLQMNSLVPEDTGVYYCVAPAWTGYGCTWGQGTQVTVSS

SEQ ID NO: 3 - protein, 132 aa, Artificial Sequence
  anti-HLA-G nanobody clone#33
MGHVQLVESGGGSVQAGGSLKLSCVTSAYTFSASGNCMGWLRQAPGKGREGIAATYTRSAKTYYADSVKGRFTISQDNAKNTVYLQMNGLKPEDTATYYCAVARCAGRPDRSTLTSFAWWGQGTQVTVSSLE

SEQ ID NO: 4 - DNA, 399 bp, Artificial Sequence
  anti-HLA-G nanobody clone#9
atgggccaggtgcagctggtggaaagcggcggcggtagtgttcaggcaggtggcagcctgcgcctgagttgtgaagcaagcggccgcacctatagcagcaattgcatgggttggtttcgccaggcaccgggcaaagaacgcgaaaatgtggcagcaatctataccggcggtgacggtattacctatgccgatagtgtgaaaggtcgttttaccattagtcaggataaactgaaaaacatgctgtatctgcagatggatagcctgaaaccggaagataccgccatgtattattgcgcagcagatccgaatcgccgccgtatgggcgttggtggcagctgcctgcgcgccaattttggcccgggcggccagggtacccaggtgaccgttagcagcctcgag

SEQ ID NO: 5 - DNA, 351 bp, Artificial Sequence
  anti-HLA-G nanobody clone#20
gaagtgcagctggttgaaagtggtggtggcagcgttcgcccgggcgaaaccttacgtctgagctgcaccgcaagtggcttcaccgtggatgatagcgatatgagctggtatcgccaggccccgggtgatgaatgtgaactggttagtagcattaccagtggtggcggcaaatattatagtcatccggtgaaaggccgcttcaccatcttccgtgataaaggtaaaaataccatgtatctgcagatgaatagcctggttccggaagataccggcgtgtattattgtgtggccccggcctggaccggctatggttgcacctggggccagggtacccaggtgaccgttagcagt

SEQ ID NO: 6 - DNA, 396 bp, Artificial Sequence
  anti-HLA-G nanobody clone#33
atgggccatgttcagctggttgaaagtggcggtggcagtgtgcaggccggtggtagtctgaaactgagctgcgttaccagcgcatataccttcagcgcaagcggtaattgtatgggctggctgcgtcaggcaccgggtaaaggccgcgaaggtattgcagccacctatacccgtagtgccaaaacctattatgcagatagtgttaaaggtcgcttcaccattagtcaggataatgcaaaaaataccgtgtatctgcagatgaatggtctgaaaccggaagataccgccacctattattgtgcagtggcacgctgtgccggtcgtccggatcgtagtaccctgaccagcttcgcctggtggggtcagggcacccaggtgaccgtgagcagcctcgag

SEQ ID NO: 7 - protein, 8 aa, Artificial Sequence
  CDR1 of anti-HLA-G nanobody clone#9
GRTYSSNC

SEQ ID NO: 8 - protein, 8 aa, Artificial Sequence
  CDR2 of anti-HLA-G nanobody clone#9
IYTGGDGI

SEQ ID NO: 9 - protein, 15 aa, Artificial Sequence
  CDR3 of anti-HLA-G nanobody clone#9
AADPNRRRMGVGGSC

SEQ ID NO: 10 - protein, 8 aa, Artificial Sequence
  CDR1 of anti-HLA-G nanobody clone#20
GFTVDDSD

SEQ ID NO: 11 - protein, 7 aa, Artificial Sequence
  CDR2 of anti-HLA-G nanobody clone#20
ITSGGGK

SEQ ID NO: 12 - protein, 11 aa, Artificial Sequence
  CDR3 of anti-HLA-G nanobody clone#20
VAPAWTGYGCT

SEQ ID NO: 13 - protein, 8 aa, Artificial Sequence
  CDR1 of anti-HLA-G nanobody clone#33
AYTFSASG

SEQ ID NO: 14 - protein, 10 aa, Artificial Sequence
  CDR2 of anti-HLA-G nanobody clone#33
AATYTRSAKT

SEQ ID NO: 15 - protein, 19 aa, Artificial Sequence
  CDR3 of anti-HLA-G nanobody clone#33
AVARCAGRPDRSTLTSFAW